European Patent Application EP 4 269 435 A1, published November 1, 2023. Title: ANTI-B7-H3 ANTIBODY AND USE THEREOF. Applicant: Innovent Biologics (Suzhou) Co., Ltd. The sequence listing filed with the application follows.

SEQUENCE LISTING (65 sequences)

SEQ ID NO: 1 - protein, 10 aa, Artificial sequence
  CDR sequence
GYTFTEYIMH

SEQ ID NO: 2 - protein, 17 aa, Artificial sequence
  CDR sequence
GINPNNGGTTYNQKFKD

SEQ ID NO: 3 - protein, 9 aa, Artificial sequence
  CDR sequence
RTPPWHFAV

SEQ ID NO: 4 - protein, 10 aa, Artificial sequence
  CDR sequence
SASSSVSYIH

SEQ ID NO: 5 - protein, 7 aa, Artificial sequence
  CDR sequence
DTSRLAS

SEQ ID NO: 6 - protein, 9 aa, Artificial sequence
  CDR sequence
QQWSSAPLT

SEQ ID NO: 7 - protein, 17 aa, Artificial sequence
  CDR sequence
GINPGTGGTTYNQKFKD

SEQ ID NO: 8 - protein, 10 aa, Artificial sequence
  CDR sequence
GYIFTSYWIH

SEQ ID NO: 9 - protein, 17 aa, Artificial sequence
  CDR sequence
RIYPGTDSTFYNEKFKG

SEQ ID NO: 10 - protein, 10 aa, Artificial sequence
  CDR sequence
ITASDWYFDV

SEQ ID NO: 11 - protein, 12 aa, Artificial sequence
  CDR sequence
SVSSSVNSNYLY

SEQ ID NO: 12 - protein, 7 aa, Artificial sequence
  CDR sequence
GTSNLAS

SEQ ID NO: 13 - protein, 9 aa, Artificial sequence
  CDR sequence
YQWSSYPFT

SEQ ID NO: 14 - protein, 17 aa, Artificial sequence
  CDR sequence
RIYPGTESTFYNEKFKG

SEQ ID NO: 15 - protein, 12 aa, Artificial sequence
  CDR sequence
SVSSSVQSNYLY

SEQ ID NO: 16 - protein, 119 aa, Artificial sequence
  VH sequence
EVQLQQSGAELVRPGASVKLSCKTSGYIFTSYWIHWIKQRSGQGLEWIARIYPGTDSTFYNEKFKGRATLTADKSSSTVYLQLNSLKSEDSAVYFCHFITASDWYFDVWGAGTTVTVSS

SEQ ID NO: 17 - protein, 108 aa, Artificial sequence
  VL sequence
DIVLTQSPAIMSASPGEKVTLTCSVSSSVNSNYLYWYQQKPGSSPKLWIYGTSNLASGVPARFSGSGSGPSYSLTISSMEAEDAASYFCYQWSSYPFTFGSGTKLEIK

SEQ ID NO: 18 - protein, 118 aa, Artificial sequence
  VH sequence
EVQLQQSVPELVKPGASVKISCKTSGYTFTEYIMHWVKQSHGKNLEWIGGINPNNGGTTYNQKFKDKATLTVDKSSSTAYMELHNLTSEDSAVYYCTRRTPPWHFAVWGAGTSLTVSS

SEQ ID NO: 19 - protein, 106 aa, Artificial sequence
  VL sequence
DIVLTQSPTIMSASPGEKVTMTCSASSSVSYIHWYQQKSGTSPKRWIFDTSRLASGVPARFSGSGSGTSYSLTISSMEAEDAATYYCQQWSSAPLTFGTGTTLELK

SEQ ID NO: 20 - protein, 119 aa, Artificial sequence
  VH sequence
QVQLVQSGAEVKKPGASVKVSCKASGYIFTSYWIHWVRQAPGQGLEWMGRIYPGTESTFYNEKFKGRVTMTRDTSTSTVYMELSSLRSEDTAVYYCHFITASDWYFDVWGQGTLVTVSS

SEQ ID NO: 21 - protein, 108 aa, Artificial sequence
  VL sequence
EIVLTQSPATLSLSPGERATLSCSVSSSVQSNYLYWYQQKPGQAPRLLIYGTSNLASGIPARFSGSGSGTDFTLTISSLEPEDFAVYYCYQWSSYPFTFGQGTKLEIK

SEQ ID NO: 22 - protein, 118 aa, Artificial sequence
  VH sequence
QVQLVQSGAEVKKPGASVKVSCKASGYTFTEYIMHWVRQAPGQRLEWMGGINPGTGGTTYNQKFKDRVTITVDTSASTAYMELSSLRSEDTAVYYCTRRTPPWHFAVWGQGTLVTVSS

SEQ ID NO: 23 - protein, 106 aa, Artificial sequence
  VL sequence
DIQLTQSPSFLSASVGDRVTITCSASSSVSYIHWYQQKPGKAPKRWIYDTSRLASGVPSRFSGSGSGTEFTLTISSLQPEDFATYYCQQWSSAPLTFGGGTKVEIK

SEQ ID NO: 24 - protein, 449 aa, Artificial sequence
  Antibody sequence
QVQLVQSGAEVKKPGASVKVSCKASGYIFTSYWIHWVRQAPGQGLEWMGRIYPGTESTFYNEKFKGRVTMTRDTSTSTVYMELSSLRSEDTAVYYCHFITASDWYFDVWGQGTLVTVSSASTKGPSVFPLAPSSKSTSGGTAALGCLVKDYFPEPVTVSWNSGALTSGVHTFPAVLQSSGLYSLSSVVTVPSSSLGTQTYICNVNHKPSNTKVDKKVEPKSCDKTHTCPPCPAPELLGGPSVFLFPPKPKDTLMISRTPEVTCVVVDVSHEDPEVKFNWYVDGVEVHNAKTKPREEQYNSTYRVVSVLTVLHQDWLNGKEYKCKVSNKALPAPIEKTISKAKGQPREPQVYTLPPSRDELTKNQVSLTCLVKGFYPSDIAVEWESNGQPENNYKTTPPVLDSDGSFFLYSKLTVDKSRWQQGNVFSCSVMHEALHNHYTQKSLSLSPGK

SEQ ID NO: 25 - protein, 215 aa, Artificial sequence
  Antibody sequence
EIVLTQSPATLSLSPGERATLSCSVSSSVQSNYLYWYQQKPGQAPRLLIYGTSNLASGIPARFSGSGSGTDFTLTISSLEPEDFAVYYCYQWSSYPFTFGQGTKLEIKRTVAAPSVFIFPPSDEQLKSGTASVVCLLNNFYPREAKVQWKVDNALQSGNSQESVTEQDSKDSTYSLSSTLTLSKADYEKHKVYACEVTHQGLSSPVTKSFNRGEC

SEQ ID NO: 26 - protein, 448 aa, Artificial sequence
  Antibody sequence
QVQLVQSGAEVKKPGASVKVSCKASGYTFTEYIMHWVRQAPGQRLEWMGGINPGTGGTTYNQKFKDRVTITVDTSASTAYMELSSLRSEDTAVYYCTRRTPPWHFAVWGQGTLVTVSSASTKGPSVFPLAPSSKSTSGGTAALGCLVKDYFPEPVTVSWNSGALTSGVHTFPAVLQSSGLYSLSSVVTVPSSSLGTQTYICNVNHKPSNTKVDKKVEPKSCDKTHTCPPCPAPELLGGPSVFLFPPKPKDTLMISRTPEVTCVVVDVSHEDPEVKFNWYVDGVEVHNAKTKPREEQYNSTYRVVSVLTVLHQDWLNGKEYKCKVSNKALPAPIEKTISKAKGQPREPQVYTLPPSRDELTKNQVSLTCLVKGFYPSDIAVEWESNGQPENNYKTTPPVLDSDGSFFLYSKLTVDKSRWQQGNVFSCSVMHEALHNHYTQKSLSLSPGK

SEQ ID NO: 27 - protein, 213 aa, Artificial sequence
  Antibody sequence
DIQLTQSPSFLSASVGDRVTITCSASSSVSYIHWYQQKPGKAPKRWIYDTSRLASGVPSRFSGSGSGTEFTLTISSLQPEDFATYYCQQWSSAPLTFGGGTKVEIKRTVAAPSVFIFPPSDEQLKSGTASVVCLLNNFYPREAKVQWKVDNALQSGNSQESVTEQDSKDSTYSLSSTLTLSKADYEKHKVYACEVTHQGLSSPVTKSFNRGEC

SEQ ID NO: 28 - protein, 449 aa, Artificial sequence
  Antibody sequence
EVQLQQSGAELVRPGASVKLSCKTSGYIFTSYWIHWIKQRSGQGLEWIARIYPGTDSTFYNEKFKGRATLTADKSSSTVYLQLNSLKSEDSAVYFCHFITASDWYFDVWGAGTTVTVSSASTKGPSVFPLAPSSKSTSGGTAALGCLVKDYFPEPVTVSWNSGALTSGVHTFPAVLQSSGLYSLSSVVTVPSSSLGTQTYICNVNHKPSNTKVDKKVEPKSCDKTHTCPPCPAPELLGGPSVFLFPPKPKDTLMISRTPEVTCVVVDVSHEDPEVKFNWYVDGVEVHNAKTKPREEQYNSTYRVVSVLTVLHQDWLNGKEYKCKVSNKALPAPIEKTISKAKGQPREPQVYTLPPSRDELTKNQVSLTCLVKGFYPSDIAVEWESNGQPENNYKTTPPVLDSDGSFFLYSKLTVDKSRWQQGNVFSCSVMHEALHNHYTQKSLSLSPGK

SEQ ID NO: 29 - protein, 215 aa, Artificial sequence
  Antibody sequence
DIVLTQSPAIMSASPGEKVTLTCSVSSSVNSNYLYWYQQKPGSSPKLWIYGTSNLASGVPARFSGSGSGPSYSLTISSMEAEDAASYFCYQWSSYPFTFGSGTKLEIKRTVAAPSVFIFPPSDEQLKSGTASVVCLLNNFYPREAKVQWKVDNALQSGNSQESVTEQDSKDSTYSLSSTLTLSKADYEKHKVYACEVTHQGLSSPVTKSFNRGEC

SEQ ID NO: 30 - protein, 448 aa, Artificial sequence
  Antibody sequence
EVQLQQSVPELVKPGASVKISCKTSGYTFTEYIMHWVKQSHGKNLEWIGGINPNNGGTTYNQKFKDKATLTVDKSSSTAYMELHNLTSEDSAVYYCTRRTPPWHFAVWGAGTSLTVSSASTKGPSVFPLAPSSKSTSGGTAALGCLVKDYFPEPVTVSWNSGALTSGVHTFPAVLQSSGLYSLSSVVTVPSSSLGTQTYICNVNHKPSNTKVDKKVEPKSCDKTHTCPPCPAPELLGGPSVFLFPPKPKDTLMISRTPEVTCVVVDVSHEDPEVKFNWYVDGVEVHNAKTKPREEQYNSTYRVVSVLTVLHQDWLNGKEYKCKVSNKALPAPIEKTISKAKGQPREPQVYTLPPSRDELTKNQVSLTCLVKGFYPSDIAVEWESNGQPENNYKTTPPVLDSDGSFFLYSKLTVDKSRWQQGNVFSCSVMHEALHNHYTQKSLSLSPGK

SEQ ID NO: 31 - protein, 213 aa, Artificial sequence
  Antibody sequence
DIVLTQSPTIMSASPGEKVTMTCSASSSVSYIHWYQQKSGTSPKRWIFDTSRLASGVPARFSGSGSGTSYSLTISSMEAEDAATYYCQQWSSAPLTFGTGTTLELKRTVAAPSVFIFPPSDEQLKSGTASVVCLLNNFYPREAKVQWKVDNALQSGNSQESVTEQDSKDSTYSLSSTLTLSKADYEKHKVYACEVTHQGLSSPVTKSFNRGEC

SEQ ID NO: 32 - protein, 534 aa, Artificial sequence
  Human 4Ig-B7H3 protein
MLRRRGSPGMGVHVGAALGALWFCLTGALEVQVPEDPVVALVGTDATLCCSFSPEPGFSLAQLNLIWQLTDTKQLVHSFAEGQDQGSAYANRTALFPDLLAQGNASLRLQRVRVADEGSFTCFVSIRDFGSAAVSLQVAAPYSKPSMTLEPNKDLRPGDTVTITCSSYQGYPEAEVFWQDGQGVPLTGNVTTSQMANEQGLFDVHSILRVVLGANGTYSCLVRNPVLQQDAHSSVTITPQRSPTGAVEVQVPEDPVVALVGTDATLRCSFSPEPGFSLAQLNLIWQLTDTKQLVHSFTEGRDQGSAYANRTALFPDLLAQGNASLRLQRVRVADEGSFTCFVSIRDFGSAAVSLQVAAPYSKPSMTLEPNKDLRPGDTVTITCSSYRGYPEAEVFWQDGQGVPLTGNVTTSQMANEQGLFDVHSVLRVVLGANGTYSCLVRNPVLQQDAHGSVTITGQPMTFPPEALWVTVGLSVCLIALLVALAFVCWRKIKQSCEEENAGAEDQDGEGEGSKTALQPLKHSDSKEDDGQEIA

SEQ ID NO: 33 - protein, 316 aa, Artificial sequence
  Human 2Ig-B7H3 protein
MLRRRGSPGMGVHVGAALGALWFCLTGALEVQVPEDPVVALVGTDATLCCSFSPEPGFSLAQLNLIWQLTDTKQLVHSFAEGQDQGSAYANRTALFPDLLAQGNASLRLQRVRVADEGSFTCFVSIRDFGSAAVSLQVAAPYSKPSMTLEPNKDLRPGDTVTITCSSYRGYPEAEVFWQDGQGVPLTGNVTTSQMANEQGLFDVHSVLRVVLGANGTYSCLVRNPVLQQDAHGSVTITGQPMTFPPEALWVTVGLSVCLIALLVALAFVCWRKIKQSCEEENAGAEDQDGEGEGSKTALQPLKHSDSKEDDGQEIA

SEQ ID NO: 34 - protein, 534 aa, Artificial sequence
  Cynomolgus monkey B7H3 protein
MLHRRGSPGMGVHVGAALGALWFCLTGALEVQVPEDPVVALVGTDATLRCSFSPEPGFSLAQLNLIWQLTDTKQLVHSFTEGRDQGSAYANRTALFLDLLAQGNASLRLQRVRVADEGSFTCFVSIRDFGSAAVSLQVAAPYSKPSMTLEPNKDLRPGDTVTITCSSYRGYPEAEVFWQDGQGAPLTGNVTTSQMANEQGLFDVHSVLRVVLGANGTYSCLVRNPVLQQDAHGSITITPQRSPTGAVEVQVPEDPVVALVGTDATLRCSFSPEPGFSLAQLNLIWQLTDTKQLVHSFTEGRDQGSAYANRTALFLDLLAQGNASLRLQRVRVADEGSFTCFVSIRDFGSAAVSLQVAAPYSKPSMTLEPNKDLRPGDTVTITCSSYRGYPEAEVFWQDGQGAPLTGNVTTSQMANEQGLFDVHSVLRVVLGANGTYSCLVRNPVLQQDAHGSVTITGQPMTFPPEALWVTVGLSVCLVALLVALAFVCWRKIKQSCEEENAGAEDQDGEGEGSKTALQPLKHSDSKEDDGQELA

SEQ ID NO: 35 - protein, 122 aa, Artificial sequence
  MGA271 VH
EVQLVESGGGLVQPGGSLRLSCAASGFTFSSFGMHWVRQAPGKGLEWVAYISSDSSAIYYADTVKGRFTISRDNAKNSLYLQMNSLRDEDTAVYYCGRGRENIYYGSRLDYWGQGTTVTVSS

SEQ ID NO: 36 - protein, 107 aa, Artificial sequence
  MGA271 VL
DIQLTQSPSFLSASVGDRVTITCKASQNVDTNVAWYQQKPGKAPKALIYSASYRYSGVPSRFSGSGSGTDFTLTISSLQPEDFATYYCQQYNNYPFTFGQGTKLEIK

SEQ ID NO: 37 - protein, 330 aa, Artificial sequence [sequence omitted]

SEQ ID NO: 38 - protein, 107 aa, Artificial sequence [sequence omitted]

SEQ ID NO: 39 - protein, 23 aa, Artificial sequence
  Primer sequence
SAGGTCCAGCTGCAGCAGYYTGG

SEQ ID NO: 40 - protein, 23 aa, Artificial sequence
  Primer sequence
CAGGTRCAGCTGAAGSAGTCAGG

SEQ ID NO: 41 - protein, 23 aa, Artificial sequence
  Primer sequence
GAKGTGCAGCTTCAGCAGTCRGG

SEQ ID NO: 42 - protein, 23 aa, Artificial sequence
  Primer sequence
GAVGTGAWGCTGGTGGAGTCTGR

SEQ ID NO: 43 - protein, 23 aa, Artificial sequence
  Primer sequence
GAAGTGCAGCTGTTGGAGACTGG

SEQ ID NO: 44 - protein, 23 aa, Artificial sequence
  Primer sequence
GAGGTTCAGCTGCAGCAGTCTGK

SEQ ID NO: 45 - protein, 23 aa, Artificial sequence
  Primer sequence
CAGGTTCACCTACAACAGTCTGG

SEQ ID NO: 46 - protein, 18 aa, Artificial sequence
  Primer sequence
CTGAGGARACGGTGACCG

SEQ ID NO: 47 - protein, 22 aa, Artificial sequence
  Primer sequence
CTGAGGAGACTGTGAGAGWGGT

SEQ ID NO: 48 - protein, 22 aa, Artificial sequence
  Primer sequence
CTGAGGAGACGGTGACTGAGGT

SEQ ID NO: 49 - protein, 22 aa, Artificial sequence
  Primer sequence
CTGCAGAGACAGTGACCAGAGT

SEQ ID NO: 50 - protein, 24 aa, Artificial sequence
  Primer sequence
GATGYTKTGATGACCCAAACTCCA

SEQ ID NO: 51 - protein, 24 aa, Artificial sequence
  Primer sequence
GATATTGTGATGACGCAGGCTGCA

SEQ ID NO: 52 - protein, 24 aa, Artificial sequence
  Primer sequence
GATATTGTGATAACCCAGGATGAA

SEQ ID NO: 53 - protein, 24 aa, Artificial sequence
  Primer sequence
GACATTGTGCTAACACAGTCTCCT

SEQ ID NO: 54 - protein, 24 aa, Artificial sequence
  Primer sequence
RACATTGTGCTSACCCAATCTCCA

SEQ ID NO: 55 - protein, 24 aa, Artificial sequence
  Primer sequence
GACATCTTGCTGACTCAGTCTCCA

SEQ ID NO: 56 - protein, 24 aa, Artificial sequence
  Primer sequence
GACATTGTGATGACCCAGTCTCAA

SEQ ID NO: 57 - protein, 24 aa, Artificial sequence
  Primer sequence
AGTATTGTGATGACCCAGACTCCC

SEQ ID NO: 58 - protein, 24 aa, Artificial sequence
  Primer sequence
GACATCMAGATGACMCAGTCTCCA

SEQ ID NO: 59 - protein, 24 aa, Artificial sequence
  Primer sequence
GAAAATGTGCTCACYCAGTCTCCA

SEQ ID NO: 60 - protein, 24 aa, Artificial sequence
  Primer sequence
GACATTGTGATGACTCAGTCTCCA

SEQ ID NO: 61 - protein, 24 aa, Artificial sequence
  Primer sequence
GACATCCAGATGATTCAGTCTCCA

SEQ ID NO: 62 - protein, 24 aa, Artificial sequence
  Primer sequence
GACATCCAGATGACCCAGTCTCCA

SEQ ID NO: 63 - protein, 24 aa, Artificial sequence
  Primer sequence
GATATCCAGATGACACAGACTACT

SEQ ID NO: 64 - protein, 24 aa, Artificial sequence
  Primer sequence
GATGTCCAGATGATTCAGTCTCCA

SEQ ID NO: 65 - protein, 20 aa, Artificial sequence
  Primer sequence
TACAGTTGGTGCAGCATCAG